European Patent Specification EP 3 759 243 B1, published September 27, 2023. Title: Methods and Compositions for Enriching Nucleic Acids. Applicant: Synpromics Limited. The sequence listing filed with the application follows.

SEQUENCE LISTING (14 sequences)

SEQ ID NO: 1 - DNA, 85 bp, Artificial Sequence
  trial single-stranded (ss) DNA oligo library
  misc_feature (38)..(62): ns indicate random nucleotides representing a random library
tcgaggccaccatgggatatcaagatcttgacgcatcnnnnnnnnnnnnnnnnnnnnnnnnnatcgaattcaccccgggtgaagc

SEQ ID NO: 2 - DNA, 21 bp, Artificial Sequence
  Blocking oligo
gatatcccatggtggcctcga

SEQ ID NO: 3 - RNA, 21 nt, Artificial Sequence
  Blocking oligo
gauaucccaugguggccucga

SEQ ID NO: 4 - DNA, 20 bp, Artificial Sequence
  5' end of general sequence layout of the finished library
tggcctaactggccggtacc

SEQ ID NO: 5 - DNA, 20 bp, Artificial Sequence
  3' end of general sequence layout of the finished library
tcgacagatctgaattccta

SEQ ID NO: 6 - DNA, 20 bp, Artificial Sequence
  blocking oligo
ggtaccggccagttaggcca

SEQ ID NO: 7 - RNA, 20 nt, Artificial Sequence
  blocking oligo
gguaccggccaguuaggcca

SEQ ID NO: 8 - DNA, 20 bp, Artificial Sequence
  3' DNA primer for primer extension
taggaattcagatctgtcga

SEQ ID NO: 9 - DNA, 109 bp, Artificial Sequence
  new trial oligo of 109 bases
  misc_feature (53)..(72): ns indicate random nucleotides and represent a random library
tgcgttggacactatcaatctaagccgtccaggacacggatctggacagcgannnnnnnnnnnnnnnnnnnntgagctctgggaggcgatcgacagatctgaattccta

SEQ ID NO: 10 - RNA, 20 nt, Artificial Sequence
  5' RNA blocking oligo
gauugauaguguccaacgca

SEQ ID NO: 11 - DNA, 20 bp, Artificial Sequence
  5' end of general sequence layout of the finished library
tgcgttggacactatcaatc

SEQ ID NO: 12 - DNA, 2689 bp, Artificial Sequence
  pSYN_ssDNA1
tcgaggccaccatgggatatcaagatcttgacgcgtaggaattcaccccgggtgaagctggcgtaatcatggtcatagctgtttcctgtgtgaaattgttatccgctcacaattccacacaacatacgagccggaagcataaagtgtaaagcctggggtgcctaatgagtgagctaactcacattaattgcgttgcgctcactgcccgctttccagtcgggaaacctgtcgtgccagctgcattaatgaatcggccaacgcgcggggagaggcggtttgcgtattgggcgctcttccgcttcctcgctcactgactcgctgcgctcggtcgttcggctgcggcgagcggtatcagctcactcaaaggcggtaatacggttatccacagaatcaggggataacgcaggaaagaacatgtgagcaaaaggccagcaaaaggccaggaaccgtaaaaaggccgcgttgctggcgtttttccataggctccgcccccctgacgagcatcacaaaaatcgacgctcaagtcagaggtggcgaaacccgacaggactataaagataccaggcgtttccccctggaagctccctcgtgcgctctcctgttccgaccctgccgcttaccggatacctgtccgcctttctcccttcgggaagcgtggcgctttctcatagctcacgctgtaggtatctcagttcggtgtaggtcgttcgctccaagctgggctgtgtgcacgaaccccccgttcagcccgaccgctgcgccttatccggtaactatcgtcttgagtccaacccggtaagacacgacttatcgccactggcagcagccactggtaacaggattagcagagcgaggtatgtaggcggtgctacagagttcttgaagtggtggcctaactacggctacactagaagaacagtatttggtatctgcgctctgctgaagccagttaccttcggaaaaagagttggtagctcttgatccggcaaacaaaccaccgctggtagcggtggtttttttgtttgcaagcagcagattacgcgcagaaaaaaaggatctcaagaagatcctttgatcttttctacggggtctgacgctcagtggaacgaaaactcacgttaagggattttggtcatgagattatcaaaaaggatcttcacctagatccttttaaattaaaaatgaagttttaaatcaatctaaagtatatatgagtaaacttggtctgacagttaccaatgcttaatcagtgaggcacctatctcagcgatctgtctatttcgttcatccatagttgcctgactccccgtcgtgtagataactacgatacgggagggcttaccatctggccccagtgctgcaatgataccgcgagacccacgctcaccggctccagatttatcagcaataaaccagccagccggaagggccgagcgcagaagtggtcctgcaactttatccgcctccatccagtctattaattgttgccgggaagctagagtaagtagttcgccagttaatagtttgcgcaacgttgttgccattgctacaggcatcgtggtgtcacgctcgtcgtttggtatggcttcattcagctccggttcccaacgatcaaggcgagttacatgatcccccatgttgtgcaaaaaagcggttagctccttcggtcctccgatcgttgtcagaagtaagttggccgcagtgttatcactcatggttatggcagcactgcataattctcttactgtcatgccatccgtaagatgcttttctgtgactggtgagtactcaaccaagtcattctgagaatagtgtatgcggcgaccgagttgctcttgcccggcgtcaatacgggataataccgcgccacatagcagaactttaaaagtgctcatcattggaaaacgttcttcggggcgaaaactctcaaggatcttaccgctgttgagatccagttcgatgtaacccactcgtgcacccaactgatcttcagcatcttttactttcaccagcgtttctgggtgagcaaaaacaggaaggcaaaatgccgcaaaaaagggaataagggcgacacggaaatgttgaatactcatactcttcctttttcaatattattgaagcatttatcagggttattgtctcatgagcggatacatatttgaatgtatttagaaaaataaacaaataggggttccgcgcacatttccccgaaaagtgccacctgacgtctaagaaaccattattatcatgacattaacctataaaaataggcgtatcacgaggccctttcgtctcgcgcgtttcggtgatgacggtgaaaacctctgacacatgcagctcccggagacggtcacagcttgtctgtaagcggatgccgggagcagacaagcccgtcagggcgcgtcagcgggtgttggcgggtgtcggggctggcttaactatgcggcatcagagcagattgtactgagagtgcaccatatgcggtgtgaaataccgcacagatgcgtaaggagaaaataccgcatcaggcgccattcgccattcaggctgcgcaactgttgggaagggcgatcggtgcgggcctcttcgctattacgccagctggcgaaagggggatgtgctgcaaggcgattaagttgggtaacgccagggttttcccagtcacgacgttgtaaaacgacggccagtg

SEQ ID NO: 13 - DNA, 2761 bp, Artificial Sequence
  pSYN_ssDNA2
cctaaattgtaagcgttaatattttgttaaaattcgcgttaaatttttgttaaatcagctcattttttaaccaataggccgaaatcggcaaaatcccttataaatcaaaagaatagaccgagatagggttgagtggccgctacagggcgctcccattcgccattcaggctgcgcaactgttgggaagggcgtttcggtgcgggcctcttcgctattacgccagctggcgaaagggggatgtgctgcaaggcgattaagttgggtaacgccagggttttcccagtcacgacgttgtaaaacgacggccagtgagcgcgacgtaatacgactcactatagggcgaattggcggaaggccgtcaaggccacgtgtcttgtccagagctcgcataataaaatatctttattttcattacatctgtgtgttggttttttgtgtggcggccgcgtggcctaactggccggtacctcgaggcgccggcgactagtcgacagatctgaattcctagagtcggggcggccggccgcttcgagcagacatgataagatacattgatgagtttggacaaaccacaactagaatgcagtgaaaaaaatgctttatttgtgaaatttgtgatgctattgctttatttgtaaccattataagctgcaataaacaagttaacaacaacaattgcattcattttatgtttcaggttcagggggaggtgtgggaggttttttaaagcaagtaaaacctctacaaatgtggtaaaatcgataaggatccgtggtacctggagcacaagactggcctcatgggccttccgctcactgcccgctttccagtcgggaaacctgtcgtgccagctgcattaacatggtcatagctgtttccttgcgtattgggcgctctccgcttcctcgctcactgactcgctgcgctcggtcgttcgggtaaagcctggggtgcctaatgagcaaaaggccagcaaaaggccaggaaccgtaaaaaggccgcgttgctggcgtttttccataggctccgcccccctgacgagcatcacaaaaatcgacgctcaagtcagaggtggcgaaacccgacaggactataaagataccaggcgtttccccctggaagctccctcgtgcgctctcctgttccgaccctgccgcttaccggatacctgtccgcctttctcccttcgggaagcgtggcgctttctcatagctcacgctgtaggtatctcagttcggtgtaggtcgttcgctccaagctgggctgtgtgcacgaaccccccgttcagcccgaccgctgcgccttatccggtaactatcgtcttgagtccaacccggtaagacacgacttatcgccactggcagcagccactggtaacaggattagcagagcgaggtatgtaggcggtgctacagagttcttgaagtggtggcctaactacggctacactagaagaacagtatttggtatctgcgctctgctgaagccagttaccttcggaaaaagagttggtagctcttgatccggcaaacaaaccaccgctggtagcggtggtttttttgtttgcaagcagcagattacgcgcagaaaaaaaggatctcaagaagatcctttgatcttttctacggggtctgacgctcagtggaacgaaaactcacgttaagggattttggtcatgagattatcaaaaaggatcttcacctagatccttttaaattaaaaatgaagttttaaatcaatctaaagtatatatgagtaaacttggtctgacagttaccaatgcttaatcagtgaggcacctatctcagcgatctgtctatttcgttcatccatagttgcctgactccccgtcgtgtagataactacgatacgggagggcttaccatctggccccagtgctgcaatgataccgcgagaaccacgctcaccggctccagatttatcagcaataaaccagccagccggaagggccgagcgcagaagtggtcctgcaactttatccgcctccatccagtctattaattgttgccgggaagctagagtaagtagttcgccagttaatagtttgcgcaacgttgttgccattgctacaggcatcgtggtgtcacgctcgtcgtttggtatggcttcattcagctccggttcccaacgatcaaggcgagttacatgatcccccatgttgtgcaaaaaagcggttagctccttcggtcctccgatcgttgtcagaagtaagttggccgcagtgttatcactcatggttatggcagcactgcataattctcttactgtcatgccatccgtaagatgcttttctgtgactggtgagtactcaaccaagtcattctgagaatagtgtatgcggcgaccgagttgctcttgcccggcgtcaatacgggataataccgcgccacatagcagaactttaaaagtgctcatcattggaaaacgttcttcggggcgaaaactctcaaggatcttaccgctgttgagatccagttcgatgtaacccactcgtgcacccaactgatcttcagcatcttttactttcaccagcgtttctgggtgagcaaaaacaggaaggcaaaatgccgcaaaaaagggaataagggcgacacggaaatgttgaatactcatactcttcctttttcaatattattgaagcatttatcagggttattgtctcatgagcggatacatatttgaatgtatttagaaaaataaacaaataggggttccgcgcacatttccccgaaaagtgcca

SEQ ID NO: 14 - DNA, 2760 bp, Artificial Sequence
  pSYN_ssDNA3
cctaaattgtaagcgttaatattttgttaaaattcgcgttaaatttttgttaaatcagctcattttttaaccaataggccgaaatcggcaaaatcccttataaatcaaaagaatagaccgagatagggttgagtggccgctacagggcgctcccattcgccattcaggctgcgcaactgttgggaagggcgtttcggtgcgggcctcttcgctattacgccagctggcgaaagggggatgtgctgcaaggcgattaagttgggtaacgccagggttttcccagtcacgacgttgtaaaacgacggccagtgagcgcgacgtaatacgactcactatagggcgaattggcggaaggccgtcaaggccacgtgtcttgtccagagctcgcataataaaatatctttattttcattacatctgtgtgttggttttttgtgtggcggccgcgtgcgttggacactatcaatctcgagcgccggcgactagtcgacagatctgaattcctagagtcggggcggccggccgcttcgagcagacatgataagatacattgatgagtttggacaaaccacaactagaatgcagtgaaaaaaatgctttatttgtgaaatttgtgatgctattgctttatttgtaaccattataagctgcaataaacaagttaacaacaacaattgcattcattttatgtttcaggttcagggggaggtgtgggaggttttttaaagcaagtaaaacctctacaaatgtggtaaaatcgataaggatccgtggtacctggagcacaagactggcctcatgggccttccgctcactgcccgctttccagtcgggaaacctgtcgtgccagctgcattaacatggtcatagctgtttccttgcgtattgggcgctctccgcttcctcgctcactgactcgctgcgctcggtcgttcgggtaaagcctggggtgcctaatgagcaaaaggccagcaaaaggccaggaaccgtaaaaaggccgcgttgctggcgtttttccataggctccgcccccctgacgagcatcacaaaaatcgacgctcaagtcagaggtggcgaaacccgacaggactataaagataccaggcgtttccccctggaagctccctcgtgcgctctcctgttccgaccctgccgcttaccggatacctgtccgcctttctcccttcgggaagcgtggcgctttctcatagctcacgctgtaggtatctcagttcggtgtaggtcgttcgctccaagctgggctgtgtgcacgaaccccccgttcagcccgaccgctgcgccttatccggtaactatcgtcttgagtccaacccggtaagacacgacttatcgccactggcagcagccactggtaacaggattagcagagcgaggtatgtaggcggtgctacagagttcttgaagtggtggcctaactacggctacactagaagaacagtatttggtatctgcgctctgctgaagccagttaccttcggaaaaagagttggtagctcttgatccggcaaacaaaccaccgctggtagcggtggtttttttgtttgcaagcagcagattacgcgcagaaaaaaaggatctcaagaagatcctttgatcttttctacggggtctgacgctcagtggaacgaaaactcacgttaagggattttggtcatgagattatcaaaaaggatcttcacctagatccttttaaattaaaaatgaagttttaaatcaatctaaagtatatatgagtaaacttggtctgacagttaccaatgcttaatcagtgaggcacctatctcagcgatctgtctatttcgttcatccatagttgcctgactccccgtcgtgtagataactacgatacgggagggcttaccatctggccccagtgctgcaatgataccgcgagaaccacgctcaccggctccagatttatcagcaataaaccagccagccggaagggccgagcgcagaagtggtcctgcaactttatccgcctccatccagtctattaattgttgccgggaagctagagtaagtagttcgccagttaatagtttgcgcaacgttgttgccattgctacaggcatcgtggtgtcacgctcgtcgtttggtatggcttcattcagctccggttcccaacgatcaaggcgagttacatgatcccccatgttgtgcaaaaaagcggttagctccttcggtcctccgatcgttgtcagaagtaagttggccgcagtgttatcactcatggttatggcagcactgcataattctcttactgtcatgccatccgtaagatgcttttctgtgactggtgagtactcaaccaagtcattctgagaatagtgtatgcggcgaccgagttgctcttgcccggcgtcaatacgggataataccgcgccacatagcagaactttaaaagtgctcatcattggaaaacgttcttcggggcgaaaactctcaaggatcttaccgctgttgagatccagttcgatgtaacccactcgtgcacccaactgatcttcagcatcttttactttcaccagcgtttctgggtgagcaaaaacaggaaggcaaaatgccgcaaaaaagggaataagggcgacacggaaatgttgaatactcatactcttcctttttcaatattattgaagcatttatcagggttattgtctcatgagcggatacatatttgaatgtatttagaaaaataaacaaataggggttccgcgcacatttccccgaaaagtgcca